European Patent Specification EP 3 766 895 B1, published July 10, 2024. Title: METHODS AND COMPOSITIONS FOR ADOPTIVE CELL THERAPY. Applicant: Juno Therapeutics, Inc. Application Not Yet Assigned. The sequence listing filed with the application follows.

SEQUENCE LISTING (159 sequences)

SEQ ID NO: 1 - protein, 12 aa, Artificial Sequence
  Synthetic
  IgG4 hinge
ESKYGPPCPPCP

SEQ ID NO: 2 - protein, 27 aa, Artificial Sequence
  Synthetic
  CD28 transmembrane domain
FWVLVVVGGVLACYSLLVTVAFIIFWV

SEQ ID NO: 3 - protein, 42 aa, Homo sapiens
  4-1BB costimulatory domain
KRGRKKLLYIFKQPFMRPVQTTQEEDGCSCRFPEEEEGGCEL

SEQ ID NO: 4 - protein, 112 aa, Artificial Sequence
  Synthetic
  CD3-zeta intracellular signaling domain
RVKFSRSADAPAYQQGQNQLYNELNLGRREEYDVLDKRRGRDPEMGGKPRRKNPQEGLYNELQKDKMAEAYSEIGMKGERRRGKGHDGLYQGLSTATKDTYDALHMQALPPR

SEQ ID NO: 5 - protein, 69 aa, Artificial Sequence
  Synthetic
  CD28-4-1BB
FWVLVVVGGVLACYSLLVTVAFIIFWVKRGRKKLLYIFKQPFMRPVQTTQEEDGCSCRFPEEEEGGCEL

SEQ ID NO: 6 - protein, 30 aa, Artificial Sequence
  Synthetic
CYSLLVTVAFIIFWVKRGRKKLLYIFKQPF

SEQ ID NO: 7 - protein, 16 aa, Artificial Sequence
  Synthetic
VAFIIFWVKRGRKKLL

SEQ ID NO: 8 - protein, 15 aa, Artificial Sequence
  Synthetic
AFIIFWVKRGRKKLL

SEQ ID NO: 9 - protein, 15 aa, Artificial Sequence
  Synthetic
FWVKRGRKKLLYIFK

SEQ ID NO: 10 - protein, 14 aa, Artificial Sequence
  Synthetic
FIIFWVKRGRKKLL

SEQ ID NO: 11 - protein, 13 aa, Artificial Sequence
  Synthetic
FIIFWVKRGRKKL

SEQ ID NO: 12 - protein, 13 aa, Artificial Sequence
  Synthetic
IIFWVKRGRKKLL

SEQ ID NO: 13 - protein, 32 aa, Artificial Sequence
  Synthetic
  Variant junction region
CYSLLVTVAFIIFWVNNKRGRKKLLYIFKQPF

SEQ ID NO: 14 - protein, 14 aa, Artificial Sequence
  Synthetic
  Variant peptide
IIFWVNNKRGRKKL

SEQ ID NO: 15 - protein, 13 aa, Artificial Sequence
  Synthetic
  Variant peptide
IIFWVNNKRGRKK

SEQ ID NO: 16 - protein, 9 aa, Artificial Sequence
  Synthetic
VAFIIFWVK

SEQ ID NO: 17 - protein, 9 aa, Artificial Sequence
  Synthetic
AFIIFWVKR

SEQ ID NO: 18 - protein, 9 aa, Artificial Sequence
  Synthetic
FIIFWVKRG

SEQ ID NO: 19 - protein, 9 aa, Artificial Sequence
  Synthetic
IIFWVKRGR

SEQ ID NO: 20 - protein, 9 aa, Artificial Sequence
  Synthetic
IFWVKRGRK

SEQ ID NO: 21 - protein, 9 aa, Artificial Sequence
  Synthetic
FWVKRGRKK

SEQ ID NO: 22 - protein, 9 aa, Artificial Sequence
  Synthetic
WVKRGRKKL

SEQ ID NO: 23 - protein, 9 aa, Artificial Sequence
  Synthetic peptide K28S
VAFIIFWVS

SEQ ID NO: 24 - protein, 9 aa, Artificial Sequence
  Synthetic peptide K28S
AFIIFWVSR

SEQ ID NO: 25 - protein, 9 aa, Artificial Sequence
  Synthetic peptide K28S
FIIFWVSRG

SEQ ID NO: 26 - protein, 9 aa, Artificial Sequence
  Synthetic peptide K28S
IIFWVSRGR

SEQ ID NO: 27 - protein, 9 aa, Artificial Sequence
  Synthetic peptide K28S
IFWVSRGRK

SEQ ID NO: 28 - protein, 9 aa, Artificial Sequence
  Synthetic peptide K28S
FWVSRGRKK

SEQ ID NO: 29 - protein, 9 aa, Artificial Sequence
  Synthetic peptide K28S
WVSRGRKKL

SEQ ID NO: 30 - protein, 9 aa, Artificial Sequence
  Synthetic peptide K28L
VAFIIFWVL

SEQ ID NO: 31 - protein, 9 aa, Artificial Sequence
  Synthetic peptide K28L
AFIIFWVLR

SEQ ID NO: 32 - protein, 9 aa, Artificial Sequence
  Synthetic peptide K28L
FIIFWVLRG

SEQ ID NO: 33 - protein, 9 aa, Artificial Sequence
  Synthetic peptide K28L
IIFWVLRGR

SEQ ID NO: 34 - protein, 9 aa, Artificial Sequence
  Synthetic peptide K28L
IFWVLRGRK

SEQ ID NO: 35 - protein, 9 aa, Artificial Sequence
  Synthetic peptide K28L
FWVLRGRKK

SEQ ID NO: 36 - protein, 9 aa, Artificial Sequence
  Synthetic peptide K28L
WVLRGRKKL

SEQ ID NO: 37 - protein, 9 aa, Artificial Sequence
  Synthetic peptide K28H
VAFIIFWVH

SEQ ID NO: 38 - protein, 9 aa, Artificial Sequence
  Synthetic peptide K28H
AFIIFWVHR

SEQ ID NO: 39 - protein, 9 aa, Artificial Sequence
  Synthetic peptide K28H
FIIFWVHRG

SEQ ID NO: 40 - protein, 9 aa, Artificial Sequence
  Synthetic peptide K28H
IIFWVHRGR

SEQ ID NO: 41 - protein, 9 aa, Artificial Sequence
  Synthetic peptide K28H
IFWVHRGRK

SEQ ID NO: 42 - protein, 9 aa, Artificial Sequence
  Synthetic peptide K28H
FWVHRGRKK

SEQ ID NO: 43 - protein, 9 aa, Artificial Sequence
  Synthetic peptide K28H
WVHRGRKKL

SEQ ID NO: 44 - protein, 9 aa, Artificial Sequence
  Synthetic peptide K28A
VAFIIFWVA

SEQ ID NO: 45 - protein, 9 aa, Artificial Sequence
  Synthetic peptide K28A
AFIIFWVAR

SEQ ID NO: 46 - protein, 9 aa, Artificial Sequence
  Synthetic peptide K28A
IIFWVARGR

SEQ ID NO: 47 - protein, 9 aa, Artificial Sequence
  Synthetic peptide K28A
IFWVARGRK

SEQ ID NO: 48 - protein, 9 aa, Artificial Sequence
  Synthetic peptide K28A
FWVARGRKK

SEQ ID NO: 49 - protein, 9 aa, Artificial Sequence
  Synthetic peptide K28A
WVARGRKKL

SEQ ID NO: 50 - protein, 9 aa, Artificial Sequence
  Synthetic peptide K28Q
VAFIIFWVQ

SEQ ID NO: 51 - protein, 9 aa, Artificial Sequence
  Synthetic peptide K28Q
AFIIFWVQR

SEQ ID NO: 52 - protein, 9 aa, Artificial Sequence
  Synthetic peptide K28Q
FIIFWVQRG

SEQ ID NO: 53 - protein, 9 aa, Artificial Sequence
  Synthetic peptide K28Q
IIFWVQRGR

SEQ ID NO: 54 - protein, 9 aa, Artificial Sequence
  Synthetic peptide K28Q
IFWVQRGRK

SEQ ID NO: 55 - protein, 9 aa, Artificial Sequence
  Synthetic peptide K28Q
FWVQRGRKK

SEQ ID NO: 56 - protein, 9 aa, Artificial Sequence
  Synthetic peptide K28Q
WVQRGRKKL

SEQ ID NO: 57 - protein, 9 aa, Artificial Sequence
  Synthetic peptide R31S
IIFWVKRGS

SEQ ID NO: 58 - protein, 9 aa, Artificial Sequence
  Synthetic peptide R31S
IFWVKRGSK

SEQ ID NO: 59 - protein, 9 aa, Artificial Sequence
  Synthetic peptide R31S
FWVKRGSKK

SEQ ID NO: 60 - protein, 9 aa, Artificial Sequence
  Synthetic peptide R31S
WVKRGSKKL

SEQ ID NO: 61 - protein, 9 aa, Artificial Sequence
  Synthetic peptide R31L
IIFWVKRGL

SEQ ID NO: 62 - protein, 9 aa, Artificial Sequence
  Synthetic peptide R31L
IFWVKRGLK

SEQ ID NO: 63 - protein, 9 aa, Artificial Sequence
  Synthetic peptide R31L
FWVKRGLKK

SEQ ID NO: 64 - protein, 9 aa, Artificial Sequence
  Synthetic peptide R31L
WVKRGLKKL

SEQ ID NO: 65 - protein, 9 aa, Artificial Sequence
  Synthetic peptide R31H
IIFWVKRGH

SEQ ID NO: 66 - protein, 9 aa, Artificial Sequence
  Synthetic peptide R31H
IFWVKRGHK

SEQ ID NO: 67 - protein, 9 aa, Artificial Sequence
  Synthetic peptide R31H
FWVKRGHKK

SEQ ID NO: 68 - protein, 9 aa, Artificial Sequence
  Synthetic peptide R31H
WVKRGHKKL

SEQ ID NO: 69 - protein, 9 aa, Artificial Sequence
  Synthetic peptide R31A
IIFWVKRGA

SEQ ID NO: 70 - protein, 9 aa, Artificial Sequence
  Synthetic peptide R31A
IFWVKRGAK

SEQ ID NO: 71 - protein, 9 aa, Artificial Sequence
  Synthetic peptide R31A
FWVKRGAKK

SEQ ID NO: 72 - protein, 9 aa, Artificial Sequence
  Synthetic peptide R31A
WVKRGAKKL

SEQ ID NO: 73 - protein, 9 aa, Artificial Sequence
  Synthetic peptide R31N
IIFWVKRGN

SEQ ID NO: 74 - protein, 9 aa, Artificial Sequence
  Synthetic peptide R31N
IFWVKRGNK

SEQ ID NO: 75 - protein, 9 aa, Artificial Sequence
  Synthetic peptide R31N
FWVKRGNKK

SEQ ID NO: 76 - protein, 9 aa, Artificial Sequence
  Synthetic peptide R31N
WVKRGNKKL

SEQ ID NO: 77 - protein, 9 aa, Artificial Sequence
  Synthetic peptide K28Q/R31S
IIFWVQRGS

SEQ ID NO: 78 - protein, 9 aa, Artificial Sequence
  Synthetic peptide K28Q/R31S
IFWVQRGSK

SEQ ID NO: 79 - protein, 9 aa, Artificial Sequence
  Synthetic peptide K28Q/R31S
FWVQRGSKK

SEQ ID NO: 80 - protein, 9 aa, Artificial Sequence
  Synthetic peptide K28Q/R31S
WVQRGSKKL

SEQ ID NO: 81 - protein, 9 aa, Artificial Sequence
  Synthetic peptide K28Q/R31A
IIFWVQRGA

SEQ ID NO: 82 - protein, 9 aa, Artificial Sequence
  Synthetic peptide K28Q/R31A
IFWVQRGAK

SEQ ID NO: 83 - protein, 9 aa, Artificial Sequence
  Synthetic peptide K28Q/R31A
FWVQRGAKK

SEQ ID NO: 84 - protein, 9 aa, Artificial Sequence
  Synthetic peptide K28Q/R31A
WVQRGAKKL

SEQ ID NO: 85 - protein, 9 aa, Artificial Sequence
  Synthetic peptide K28Q/R31N
IIFWVQRGN

SEQ ID NO: 86 - protein, 9 aa, Artificial Sequence
  Synthetic peptide K28Q/R31N
IFWVQRGNK

SEQ ID NO: 87 - protein, 9 aa, Artificial Sequence
  Synthetic peptide K28Q/R31N
FWVQRGNKK

SEQ ID NO: 88 - protein, 9 aa, Artificial Sequence
  Synthetic peptide K28Q/R31N
WVQRGNKKL

SEQ ID NO: 89 - protein, 9 aa, Artificial Sequence
  Synthetic peptide L34S
WVKRGRKKS

SEQ ID NO: 90 - protein, 9 aa, Artificial Sequence
  Synthetic peptide L34A
WVKRGRKKA

SEQ ID NO: 91 - protein, 9 aa, Artificial Sequence
  Synthetic peptide K28Q/L34S
WVQRGNKKS

SEQ ID NO: 92 - protein, 9 aa, Artificial Sequence
  Synthetic peptide K28Q/L34A
WVQRGNKKA

SEQ ID NO: 93 - protein, 255 aa, Homo sapiens
  4-1BB
MGNSCYNIVATLLLVLNFERTRSLQDPCSNCPAGTFCDNNRNQICSPCPPNSFSSAGGQRTCDICRQCKGVFRTRKECSSTSNAECDCTPGFHCLGAGCSMCEQDCKQGQELTKKGCKDCCFGTFNDQKRGICRPWTNCSLDGKSVLVNGTKERDVVCGPSPADLSPGASSVTPPAPAREPGHSPQIISFFLALTSTALLFLLFFLTLRFSVVKRGRKKLLYIFKQPFMRPVQTTQEEDGCSCRFPEEEEGGCEL

SEQ ID NO: 94 - protein, 255 aa, Homo sapiens; identical to SEQ ID NO: 93
  CD28

SEQ ID NO: 95 - protein, 164 aa, Homo sapiens
  CD3 zeta chain
MKWKALFTAAILQAQLPITEAQSFGLLDPKLCYLLDGILFIYGVILTALFLRVKFSRSADAPAYQQGQNQLYNELNLGRREEYDVLDKRRGRDPEMGGKPQRRKNPQEGLYNELQKDKMAEAYSEIGMKGERRRGKGHDGLYQGLSTATKDTYDALHMQALPPR

SEQ ID NO: 96 - protein, 14 aa, Artificial Sequence
  Synthetic
FIIFWVNNKRGRKK

SEQ ID NO: 97 - protein, 14 aa, Artificial Sequence
  Synthetic
IFWVNNKRGRKKLL

SEQ ID NO: 98 - protein, 14 aa, Artificial Sequence
  Synthetic
FIIFWVNNKRGRKK

SEQ ID NO: 99 - protein, 14 aa, Artificial Sequence
  Synthetic
IFWVNNKRGRKKLL

SEQ ID NO: 100 - protein, 9 aa, Artificial Sequence
  Synthetic peptide K28R
VAFIIFWVR

SEQ ID NO: 101 - protein, 9 aa, Artificial Sequence
  Synthetic peptide K28R
AFIIFWVRR

SEQ ID NO: 102 - protein, 9 aa, Artificial Sequence
  Synthetic peptide K28A
FIIFWVARG

SEQ ID NO: 103 - protein, 28 aa, Homo sapiens
  CD28 transmembrane domain
MFWVLVVVGGVLACYSLLVTVAFIIFWV

SEQ ID NO: 104 - protein, 66 aa, Homo sapiens
  CD28
IEVMYPPPYLDNEKSNGTIIHVKGKHLCPSPLFPGPSKPFWVLVVVGGVLACYSLLVTVAFIIFWV

SEQ ID NO: 105 - protein, 112 aa, Homo sapiens
  CD3 zeta
RVKFSRSAEPPAYQQGQNQLYNELNLGRREEYDVLDKRRGRDPEMGGKPRRKNPQEGLYNELQKDKMAEAYSEIGMKGERRRGKGHDGLYQGLSTATKDTYDALHMQALPPR

SEQ ID NO: 106 - DNA, 36 bp, Homo sapiens
  spacer (IgG4hinge)
gaatctaagtacggaccgccctgccccccttgccct

SEQ ID NO: 107 - protein, 119 aa, Homo sapiens
  Hinge-CH3 spacer
ESKYGPPCPPCPGQPREPQVYTLPPSQEEMTKNQVSLTCLVKGFYPSDIAVEWESNGQPENNYKTTPPVLDSDGSFFLYSRLTVDKSRWQEGNVFSCSVMHEALHNHYTQKSLSLSLGK

SEQ ID NO: 108 - protein, 229 aa, Homo sapiens
  Hinge-CH2-CH3 spacer
ESKYGPPCPPCPAPEFLGGPSVFLFPPKPKDTLMISRTPEVTCVVVDVSQEDPEVQFNWYVDGVEVHNAKTKPREEQFNSTYRVVSVLTVLHQDWLNGKEYKCKVSNKGLPSSIEKTISKAKGQPREPQVYTLPPSQEEMTKNQVSLTCLVKGFYPSDIAVEWESNGQPENNYKTTPPVLDSDGSFFLYSRLTVDKSRWQEGNVFSCSVMHEALHNHYTQKSLSLSLGK

SEQ ID NO: 109 - protein, 282 aa, Homo sapiens
  IgD-hinge-Fc
RWPESPKAQASSVPTAQPQAEGSLAKATTAPATTRNTGRGGEEKKKEKEKEEQEERETKTPECPSHTQPLGVYLLTPAVQDLWLRDKATFTCFVVGSDLKDAHLTWEVAGKVPTGGVEEGLLERHSNGSQSQHSRLTLPRSLWNAGTSVTCTLNHPSLPPQRLMALREPAAQAPVKLSLNLLASSDPPEAASWLLCEVSGFSPPNILLMWLEDQREVNTSGFAPARPPPQPGSTTFWAWSVLRVPAPPSPQPATYTCVVSHEDSRTLLNASRSLEVSYVTDH

SEQ ID NO: 110 - protein, 24 aa, Artificial Sequence
  Synthetic
  T2A
LEGGGEGRGSLLTCGDVEENPGPR

SEQ ID NO: 111 - protein, 357 aa, Artificial Sequence
  Synthetic
  tEGFR
MLLLVTSLLLCELPHPAFLLIPRKVCNGIGIGEFKDSLSINATNIKHFKNCTSISGDLHILPVAFRGDSFTHTPPLDPQELDILKTVKEITGFLLIQAWPENRTDLHAFENLEIIRGRTKQHGQFSLAVVSLNITSLGLRSLKEISDGDVIISGNKNLCYANTINWKKLFGTSGQKTKIISNRGENSCKATGQVCHALCSPEGCWGPEPRDCVSCRNVSRGRECVDKCNLLEGEPREFVENSECIQCHPECLPQAMNITCTGRGPDNCIQCAHYIDGPHCVKTCPAGVMGENNTLVWKYADAGHVCHLCHPNCTYGCTGPGLEGCPTNGPKIPSIATGMVGALLLLLVVALGIGLFM

SEQ ID NO: 112 - protein, 41 aa, Homo sapiens
  CD28 cytoplasmic domain
RSKRSRLLHSDYMNMTPRRPGPTRKHYQPYAPPRDFAAYRS

SEQ ID NO: 113 - protein, 41 aa, Homo sapiens
  CD28 cytoplasmic domain
RSKRSRGGHSDYMNMTPRRPGPTRKHYQPYAPPRDFAAYRS

SEQ ID NO: 114 - protein, 69 aa, Artificial Sequence
  Synthetic K28A
FWVLVVVGGVLACYSLLVTVAFIIFWVARGRKKLLYIFKQPFMRPVQTTQEEDGCSCRFPEEEEGGCEL

SEQ ID NO: 115 - protein, 69 aa, Artificial Sequence
  Synthetic K28H
FWVLVVVGGVLACYSLLVTVAFIIFWVHRGRKKLLYIFKQPFMRPVQTTQEEDGCSCRFPEEEEGGCEL

SEQ ID NO: 116 - protein, 69 aa, Artificial Sequence
  Synthetic K28L
FWVLVVVGGVLACYSLLVTVAFIIFWVLRGRKKLLYIFKQPFMRPVQTTQEEDGCSCRFPEEEEGGCEL

SEQ ID NO: 117 - protein, 69 aa, Artificial Sequence
  Synthetic K28Q
FWVLVVVGGVLACYSLLVTVAFIIFWVQRGRKKLLYIFKQPFMRPVQTTQEEDGCSCRFPEEEEGGCEL

SEQ ID NO: 118 - protein, 69 aa, Artificial Sequence
  Synthetic K28S
FWVLVVVGGVLACYSLLVTVAFIIFWVSRGRKKLLYIFKQPFMRPVQTTQEEDGCSCRFPEEEEGGCEL

SEQ ID NO: 119 - protein, 69 aa, Artificial Sequence
  Synthetic R31A
FWVLVVVGGVLACYSLLVTVAFIIFWVKRGAKKLLYIFKQPFMRPVQTTQEEDGCSCRFPEEEEGGCEL

SEQ ID NO: 120 - protein, 69 aa, Artificial Sequence
  Synthetic R31H
FWVLVVVGGVLACYSLLVTVAFIIFWVKRGHKKLLYIFKQPFMRPVQTTQEEDGCSCRFPEEEEGGCEL

SEQ ID NO: 121 - protein, 69 aa, Artificial Sequence
  Synthetic R31L
FWVLVVVGGVLACYSLLVTVAFIIFWVKRGLKKLLYIFKQPFMRPVQTTQEEDGCSCRFPEEEEGGCEL

SEQ ID NO: 122 - protein, 69 aa, Artificial Sequence
  Synthetic R31N
FWVLVVVGGVLACYSLLVTVAFIIFWVKRGNKKLLYIFKQPFMRPVQTTQEEDGCSCRFPEEEEGGCEL

SEQ ID NO: 123 - protein, 69 aa, Artificial Sequence
  Synthetic L34A
FWVLVVVGGVLACYSLLVTVAFIIFWVKRGRKKALYIFKQPFMRPVQTTQEEDGCSCRFPEEEEGGCEL

SEQ ID NO: 124 - protein, 69 aa, Artificial Sequence
  Synthetic L34S
FWVLVVVGGVLACYSLLVTVAFIIFWVKRGRKKSLYIFKQPFMRPVQTTQEEDGCSCRFPEEEEGGCEL

SEQ ID NO: 125 - protein, 69 aa, Artificial Sequence
  Synthetic K28Q/R31A
FWVLVVVGGVLACYSLLVTVAFIIFWVQRGAKKLLYIFKQPFMRPVQTTQEEDGCSCRFPEEEEGGCEL

SEQ ID NO: 126 - protein, 69 aa, Artificial Sequence
  Synthetic K28Q/R31N
FWVLVVVGGVLACYSLLVTVAFIIFWVQRGNKKLLYIFKQPFMRPVQTTQEEDGCSCRFPEEEEGGCEL

SEQ ID NO: 127 - protein, 69 aa, Artificial Sequence
  Synthetic K28Q/R31S
FWVLVVVGGVLACYSLLVTVAFIIFWVQRGSKKLLYIFKQPFMRPVQTTQEEDGCSCRFPEEEEGGCEL

SEQ ID NO: 128 - protein, 69 aa, Artificial Sequence
  Synthetic K28Q/L34A
FWVLVVVGGVLACYSLLVTVAFIIFWVQRGRKKALYIFKQPFMRPVQTTQEEDGCSCRFPEEEEGGCEL

SEQ ID NO: 129 - protein, 69 aa, Artificial Sequence
  Synthetic K28Q/L34S
FWVLVVVGGVLACYSLLVTVAFIIFWVQRGRKKSLYIFKQPFMRPVQTTQEEDGCSCRFPEEEEGGCEL

SEQ ID NO: 130 - protein, 69 aa, Artificial Sequence
  Synthetic R31N/L34A
FWVLVVVGGVLACYSLLVTVAFIIFWVKRGNKKALYIFKQPFMRPVQTTQEEDGCSCRFPEEEEGGCEL

SEQ ID NO: 131 - protein, 69 aa, Artificial Sequence
  Synthetic R31N/L34S
FWVLVVVGGVLACYSLLVTVAFIIFWVKRGNKKSLYIFKQPFMRPVQTTQEEDGCSCRFPEEEEGGCEL

SEQ ID NO: 132 - protein, 69 aa, Artificial Sequence
  Synthetic K28Q/R31N/L34A
FWVLVVVGGVLACYSLLVTVAFIIFWVQRGNKKALYIFKQPFMRPVQTTQEEDGCSCRFPEEEEGGCEL

SEQ ID NO: 133 - protein, 69 aa, Artificial Sequence
  Synthetic K28Q/R31N/L34S
FWVLVVVGGVLACYSLLVTVAFIIFWVQRGNKKSLYIFKQPFMRPVQTTQEEDGCSCRFPEEEEGGCEL

SEQ ID NO: 134 - protein, 71 aa, Artificial Sequence
  Synthetic
  NN Insertion
FWVLVVVGGVLACYSLLVTVAFIIFWVNNKRGRKKLLYIFKQPFMRPVQTTQEEDGCSCRFPEEEEGGCEL

SEQ ID NO: 135 - protein, 70 aa, Artificial Sequence
  Synthetic
MFWVLVVVGGVLACYSLLVTVAFIIFWVKRGRKKLLYIFKQPFMRPVQTTQEEDGCSCRFPEEEEGGCEL

SEQ ID NO: 136 - protein, 108 aa, Artificial Sequence
  Synthetic
IEVMYPPPYLDNEKSNGTIIHVKGKHLCPSPLFPGPSKPFWVLVVVGGVLACYSLLVTVAFIIFWVKRGRKKLLYIFKQPFMRPVQTTQEEDGCSCRFPEEEEGGCEL

SEQ ID NO: 137 - protein, 26 aa, Artificial Sequence
  Synthetic
  junction region
SLLVTVAFIIFWVKRGRKKLLYIFKQ

SEQ ID NO: 138 - protein, 26 aa, Artificial Sequence
  Synthetic
  junction region K14A
SLLVTVAFIIFWVARGRKKLLYIFKQ

SEQ ID NO: 139 - protein, 26 aa, Artificial Sequence
  Synthetic
  junction region K14H
SLLVTVAFIIFWVHRGRKKLLYIFKQ

SEQ ID NO: 140 - protein, 26 aa, Artificial Sequence
  Synthetic
  junction region K14L
SLLVTVAFIIFWVLRGRKKLLYIFKQ

SEQ ID NO: 141 - protein, 26 aa, Artificial Sequence
  Synthetic
  junction region K14Q
SLLVTVAFIIFWVQRGRKKLLYIFKQ

SEQ ID NO: 142 - protein, 26 aa, Artificial Sequence
  Synthetic
  junction region K14S
SLLVTVAFIIFWVSRGRKKLLYIFKQ

SEQ ID NO: 143 - protein, 26 aa, Artificial Sequence
  Synthetic
  junction region R17A
SLLVTVAFIIFWVKRGAKKLLYIFKQ

SEQ ID NO: 144 - protein, 26 aa, Artificial Sequence
  Synthetic
  junction region R17H
SLLVTVAFIIFWVKRGHKKLLYIFKQ

SEQ ID NO: 145 - protein, 26 aa, Artificial Sequence
  Synthetic
  junction region R17L
SLLVTVAFIIFWVKRGLKKLLYIFKQ

SEQ ID NO: 146 - protein, 26 aa, Artificial Sequence
  Synthetic
  junction region R17N
SLLVTVAFIIFWVKRGNKKLLYIFKQ

SEQ ID NO: 147 - protein, 26 aa, Artificial Sequence
  Synthetic
  junction region L20A
SLLVTVAFIIFWVKRGRKKALYIFKQ

SEQ ID NO: 148 - protein, 26 aa, Artificial Sequence
  Synthetic
  junction region L20S
SLLVTVAFIIFWVKRGRKKSLYIFKQ

SEQ ID NO: 149 - protein, 26 aa, Artificial Sequence
  Synthetic
  junction region K14Q/R17A
SLLVTVAFIIFWVQRGAKKLLYIFKQ

SEQ ID NO: 150 - protein, 26 aa, Artificial Sequence
  Synthetic
  junction region K14Q/R17N
SLLVTVAFIIFWVQRGNKKLLYIFKQ

SEQ ID NO: 151 - protein, 26 aa, Artificial Sequence
  Synthetic
  junction region K14Q/R17S
SLLVTVAFIIFWVQRGSKKLLYIFKQ

SEQ ID NO: 152 - protein, 26 aa, Artificial Sequence
  Synthetic
  junction region K14Q/L20A
SLLVTVAFIIFWVQRGRKKALYIFKQ

SEQ ID NO: 153 - protein, 26 aa, Artificial Sequence
  Synthetic
  junction region K14Q/L20S
SLLVTVAFIIFWVQRGRKKSLYIFKQ

SEQ ID NO: 154 - protein, 26 aa, Artificial Sequence
  Synthetic
  junction region R17N/L20A
SLLVTVAFIIFWVKRGNKKALYIFKQ

SEQ ID NO: 155 - protein, 26 aa, Artificial Sequence
  Synthetic
  junction region R17N/L20S
SLLVTVAFIIFWVKRGNKKSLYIFKQ

SEQ ID NO: 156 - protein, 26 aa, Artificial Sequence
  Synthetic
  junction region K14Q/R17N/L20A
SLLVTVAFIIFWVQRGNKKALYIFKQ

SEQ ID NO: 157 - protein, 26 aa, Artificial Sequence
  Synthetic
  junction region K14Q/R17N/L20S
SLLVTVAFIIFWVQRGNKKSLYIFKQ

SEQ ID NO: 158 - DNA, 36 bp, Homo sapiens; identical to SEQ ID NO: 106
  spacer (IgG4hinge)

SEQ ID NO: 159 - protein, 112 aa, Artificial Sequence
  Synthetic
  CD3 Zeta
RVKFSRSADAPAYKQGQNQLYNELNLGRREEYDVLDKRRGRDPEMGGKPRRKNPQEGLYNELQKDKMAEAYSEIGMKGERRRGKGHDGLYQGLSTATKDTYDALHMQALPPR